European Patent Application EP 4 582 096 A1, published July 9, 2025. Title: 재조합 안정화 갈렉틴 9 단백질을 포함하는 루푸스 예방 또는 치료용 조성물. Applicant: (주)지바이오로직스. Application KR. The sequence listing filed with the application follows.

SEQUENCE LISTING (4 sequences)

SEQ ID NO: 1 - protein, 284 aa, synthetic construct
  REGION 1..284: note = sGal-9
MAFSGSQAPYLSPAVPFSGTIQGGLQDGLQITVNGTVLSSSGTRFAVNFQTGFSGNDIAFHFNPRFEDGGYVVCNTRQNGSWGPEERKTHMPFQKGMPFDLCFLVQSSDFKVMVNGILFVQYFHRVPFHRVDTISVNGSVQLSYISFQHPPYPMPFITTILGGLYPSKSILLSGTVLPSAQRFHINLCSGNHIAFHLNPRFDENAVVRNTQIDNSWGSEERSLPRKMPFVRGQSFSVWILCEAHCLKVAVDGQHLFEYYHRLRNLPTINRLEVGGDIQLTHVQT

SEQ ID NO: 2 - protein, 146 aa, synthetic construct
  REGION 1..146: note = CCRD
TPAIPPMMYPHPAYPMPFITTILGGLYPSKSILLSGTVLPSAQRFHINLCSGNHIAFHLNPRFDENAVVRNTQIDNSWGSEERSLPRKMPFVRGQSFSVWILCEAHCLKVAVDGQHLFEYYHRLRNLPTINRLEVGGDIQLTHVQT

SEQ ID NO: 3 - protein, 10 aa, synthetic construct
  REGION 1..10: note = CCRD 1-10
TPAIPPMMYP

SEQ ID NO: 4 - protein, 283 aa, synthetic construct
  REGION 1..283: note = sGal-9_Met_del
AFSGSQAPYLSPAVPFSGTIQGGLQDGLQITVNGTVLSSSGTRFAVNFQTGFSGNDIAFHFNPRFEDGGYVVCNTRQNGSWGPEERKTHMPFQKGMPFDLCFLVQSSDFKVMVNGILFVQYFHRVPFHRVDTISVNGSVQLSYISFQHPPYPMPFITTILGGLYPSKSILLSGTVLPSAQRFHINLCSGNHIAFHLNPRFDENAVVRNTQIDNSWGSEERSLPRKMPFVRGQSFSVWILCEAHCLKVAVDGQHLFEYYHRLRNLPTINRLEVGGDIQLTHVQT